European Patent Application EP 4 219 547 A2, published August 2, 2023. Title: FACTOR IX POLYPEPTIDE MUTANT, ITS USES AND METHOD FOR ITS PRODUCTION. Applicant: UniQure N.V. Application EP. The sequence listing filed with the application follows.

SEQUENCE LISTING (13 sequences)

SEQ ID NO: 1 - protein, 461 aa, Homo sapiens [sequence omitted]

SEQ ID NO: 2 - protein, 415 aa, Homo sapiens
  PEPTIDE 1..415
  SITE 338: note = RESIDUE CORRESPONDING TO 384 OF SEQ ID No. 2
  SITE 338: note = RESIDUE MUTATED IN THE CLAIMED INVENTION
YNSGKLEEFVQGNLERECMEEKCSFEEAREVFENTERTTEFWKQYVDGDQCESNPCLNGGSCKDDINSYECWCPFGFEGKNCELDVTCNIKNGRCEQFCKNSADNKVVCSCTEGYRLAENQKSCEPAVPFPCGRVSVSQTSKLTRAETVFPDVDYVNSTEAETILDNITQSTQSFNDFTRVVGGEDAKPGQFPWQVVLNGKVDAFCGGSIVNEKWIVTAAHCVETGVKITVVAGEHNIEETEHTEQKRNVIRIIPHHNYNAAINKYNHDIALLELDEPLVLNSYVTPICIADKEYTNIFLKFGSGYVSGWGRVFHKGRSALVLQYLRVPLVDRATCLRSTKFTIYNNMFCAGFHEGGRDSCQGDSGGPHVTEVEGTSFLTGIISWGEECAMKGKYGIYTKVSRYVNWIKEKTKLT

SEQ ID NO: 3 - RNA, 1381 nt, Homo sapiens
  source 1..1381: mol_type = unassigned RNA
tgcagcgcgtgaacatgatcatggcagaatcaccaggcctcatcaccatctgccttttaggatatctactcagtgctgaatgtacagtttttcttgatcatgaaaacgccaacaaaattctgaatcggccaaagaggtataattcaggtaaattggaagagtttgttcaagggaaccttgagagagaatgtatggaagaaaagtgtagttttgaagaagcacgagaagtttttgaaaacactgaaagaacaactgaattttggaagcagtatgttgatggagatcagtgtgagtccaatccatgtttaaatggcggcagttgcaaggatgacattaattcctatgaatgttggtgtccctttggatttgaaggaaagaactgtgaattagatgtaacatgtaacattaagaatggcagatgcgagcagttttgtaaaaatagtgctgataacaaggtggtttgctcctgtactgagggatatcgacttgcagaaaaccagaagtcctgtgaaccagcagtgccatttccatgtggaagagtttctgtttcacaaacttctaagctcacccgtgctgaggctgtttttcctgatgtggactatgtaaattctactgaagctgaaaccattttggataacatcactcaaagcacccaatcatttaatgacttcactcgggttgttggtggagaagatgccaaaccaggtcaattcccttggcaggttgttttgaatggtaaagttgatgcattctgtggaggctctatcgttaatgaaaaatggattgtaactgctgcccactgtgttgaaactggtgttaaaattacagttgtcgcaggtgaacataatattgaggagacagaacatacagagcaaaagcgaaatgtgattcgaattattcctcaccacaactacaatgcagctattaataagtacaaccatgacattgcccttctggaactggacgaacccttagtgctaaacagctacgttacacctatttgcattgctgacaaggaatacacgaacatcttcctcaaatttggatctggctatgtaagtggctggggaagagtcttccacaaagggagatcagctttagttcttcagtaccttagagttccacttgttgaccgagccacatgtcttcgatctacaaagttcaccatctataacaacatgttctgtgctggcttccatgaaggaggtagagattcatgtcaaggagatagtgggggaccccatgttactgaagtggaagggaccagtttcttaactggaattattagctggggtgaagagtgtgcaatgaaaggcaaatatggaatatataccaaggtatcccggtatgtcaactggattaaggaaaaaacaaagctcac

SEQ ID NO: 4 - RNA, 1243 nt, Homo sapiens
  source 1..1243: mol_type = unassigned RNA
ataattcaggtaaattggaagagtttgttcaagggaaccttgagagagaatgtatggaagaaaagtgtagttttgaagaagcacgagaagtttttgaaaacactgaaagaacaactgaattttggaagcagtatgttgatggagatcagtgtgagtccaatccatgtttaaatggcggcagttgcaaggatgacattaattcctatgaatgttggtgtccctttggatttgaaggaaagaactgtgaattagatgtaacatgtaacattaagaatggcagatgcgagcagttttgtaaaaatagtgctgataacaaggtggtttgctcctgtactgagggatatcgacttgcagaaaaccagaagtcctgtgaaccagcagtgccatttccatgtggaagagtttctgtttcacaaacttctaagctcacccgtgctgaggctgtttttcctgatgtggactatgtaaattctactgaagctgaaaccattttggataacatcactcaaagcacccaatcatttaatgacttcactcgggttgttggtggagaagatgccaaaccaggtcaattcccttggcaggttgttttgaatggtaaagttgatgcattctgtggaggctctatcgttaatgaaaaatggattgtaactgctgcccactgtgttgaaactggtgttaaaattacagttgtcgcaggtgaacataatattgaggagacagaacatacagagcaaaagcgaaatgtgattcgaattattcctcaccacaactacaatgcagctattaataagtacaaccatgacattgcccttctggaactggacgaacccttagtgctaaacagctacgttacacctatttgcattgctgacaaggaatacacgaacatcttcctcaaatttggatctggctatgtaagtggctggggaagagtcttccacaaagggagatcagctttagttcttcagtaccttagagttccacttgttgaccgagccacatgtcttcgatctacaaagttcaccatctataacaacatgttctgtgctggcttccatgaaggaggtagagattcatgtcaaggagatagtgggggaccccatgttactgaagtggaagggaccagtttcttaactggaattattagctggggtgaagagtgtgcaatgaaaggcaaatatggaatatataccaaggtatcccggtatgtcaactggattaaggaaaaaacaaagctcac

SEQ ID NO: 5 - DNA, 5280 bp, Homo sapiens
  misc_feature 600..601: note = /note="intron between positions 600-601 not shown, approx length 5400bp" /note="position 601 corresponds to position 6000 in Anson et al paper"
  misc_feature 1200..1201: note = /note="Intron between position 1200 and 1201, approx length 3960 bp" /note="position 1200 corresponds to position 6600 in Fig 4 of Anson et al paper, position 1201 corresponds to position 10560 in Fig 4 of Anson et al."
  misc_feature 1440..1441: note = /note="Intron present between positions 1440 and 1441, approx length 7320 bp" /note="position 1440 corresponds to 10800 in Fig 4 of Anson et al, position 1441 corresponds to 18120 in Fig 4 of Anson et al"
  misc_feature 1800..1801: note = /note="Intron between positions 1880-1801, approx length 2400 bp " /note="position 1800 corresponds to position 18480 in Fig 4 of Anson et al, position 1801 corresponds to position 20880 of Anson et al"
  misc_feature 2160..2161: note = /note="Intron between 2160 and 2161, approx length 9960 bp" /note="position 2160 corresponds to 21240 in Fig 4 of Anson et al, position 2161 correspnds to 31080 of Fig 4 of Anson et al"
  misc_feature 3398: note = /note="equivalent to position 32318 in Figure 4 of Anson et al paper"
  source 1..5280: mol_type = genomic DNA
  CDS 325..411: note = /transl_table=1
  CDS 776..940: note = /transl_table=1
  CDS 1129..1152: note = /transl_table=1
  CDS 1264..1377: note = /transl_table=1
  CDS 1582..1710: note = /transl_table=1
  CDS 1881..2084: note = /transl_table=1
  CDS 2303..2416: note = /transl_table=1
  CDS 3085..3630: note = /transl_table=1
ctctctgacaaagatacggtgggtcccactgatgaactgtgctgccacagtaaatgtagccactatgcctatctccattctgaagatgtgtcacttcctgtttcagactcaaatcagccacagtggcagaagcccacagaatcagaggtgaaatttaataatgaccactgcccattctcttcacttgtcccaagaggccattggaaatagtccaaagacccattgagggagatggacattatttcccagaagtaaatacagctcagcttgtactttggtacaactaatcgaccttaccactttcacaacttgctagcagaggttatgcagcgcgtgaacatgatcatggcagaatcaccaggcctcatcaccatctgccttttaggatatctactcagtgctgaatgtacaggtttgtttccttttttaaaatacattgagtatgcttgccttttagatatagaaatatctgatgctgtcttcttcactaaattttgattacatgatttgacagcaatattgaagagtctaacagccagcacgcaggttggtaagtactggttctttgttagctaggttttcttcttcttcatttttaaaaatctccatgtgtatacagtactgtgggaacatcacagattttggctcctatgccctaaagagaaattggctttcagattatttggattaaaaacaaagactttcttaagagatgtaaaattttcatgatgttttcttttttgctaaaactaaagaattattcttttacatttcagtttttcttgatcatgaaaacgccaacaaaattctgaatcggccaaagaggtataattcaggtaaattggaagagtttgttcaagggaaccttgagagagaatgtatggaagaaaagtgtagttttgaagaagcacgagaagtttttgaaaacactgaaagaacagtgagtatttccacataatacccttcagatgcagagcatagaatagaaaatctttaaaaagacacttctctttaaaattttaaagcatccatatatatttatgtatgttaaatgttataaaagataggaaatcaataccaaaacactttagatattaccgttaatttgtcttcttttattctttatagactgaattttggaagcagtatgttggtaagcaattcattttatcctctagctaatatatgaaacatatgagacaggggaggaccgggcattctaagcagtttacgtgccaattcaatttcttaacctatctcaaagatggagatcagtgtgagtccaatccatgtttaaatggcggcagttgcaaggatgacattaattcctatgaatgttggtgtccctttggatttgaaggaaagaactgtgaattaggtaagtaactattttttgaatactcatggttcaaagtttccctctgaaacaagttgaaactgaaaatttctctccccaacgtatattgggggcaacatgaatgcccccaatgtatatttgacccatacatgagtcagtagttccatgtactttttagaaatgcatgttaaatgatgctgttactgtctattttgcttcttttagatgtaacatgtaacattaagaatggcagatgcgagcagttttgtaaaaatagtgctgataacaaggtggtttgctcctgtactgagggatatcgacttgcagaaaaccagaagtcctgtgaaccagcaggtcataatctgaataagattttttaaagaaaatctgtatctgaaacttcagcattttaacaaacctacataattttaattcctacttgacctcaatctcaatttttgtaatacatgttccatttgccaatgagaaatatcaggttactaatttttcttctatttttctagtgccatttccatgtggaagagtttctgtttcacaaacttctaagctcacccgtgctgaggctgtttttcctgatgtggactatgtaaattctactgaagctgaaaccattttggataacatcactcaaagcacccaatcatttaatgacttcactcgggttgttggtggagaagatgccaaaccaggtcaattcccttggcaggtactttatactgatggtgtgtcaaaactggagctcagctggcaagacacaggccaggtgggagactgaggctattaaagctcacatttccagaaacattccatttctgccagcacctagaagccaatattttgcctattcctgtaaccagcacacatatttatttttttctagatcaaatgtattatgcagtaagagtcttaattttgttttcacaggttgttttgaatggtaaagttgatgcattctgtggaggctctatcgttaatgaaaaatggattgtaactgctgcccactgtgttgaaactggtgttaaaattacagttgtcgcaggtaaatacacagaaagaataataatctgcagcaccactagctctttaatatgattggtacaccatattttactaaggtctaataaaattgttgttgaataaattgggctaaaggcagaagggtcataatttcagaacccacgtcgcaccgtcctccaagcatccatagttcttttgatatacccctattatcactcatttcagtgaggtacaattagttcttgatgtagccatttccataccagaaggccttcccaaaaatcagtgtcatgtcaccgatccttttatctctggtgcttggcacaacctgtagcaggtcctcagaaaacaaacatttgaattaatggccaaatgagtttgtgctcaaaaaaggggtgaggatacttgaaatttggaaaatctaggataattcatgactagtggattcattatcaccaatgaaaggcttataacagcatgagtgaacagaaccatctctatgatagtcctgaatggctttttggtctgaaaaatatgcattggctctcattacatttaaccaaaattatcacaatataagaatgagatctttaacattgccaattaggtcagtggtcccaagtagtcacttagaaaatctgtgtatgtgaaatactgtttgtgacttaaaatgaaatttatttttaataggtgaacataatattgaggagacagaacatacagagcaaaagcgaaatgtgattcgaattattcctcaccacaactacaatgcagctattaataagtacaaccatgacattgcccttctggaactggacgaacccttagtgctaaacagctacgttacacctatttgcattgctgacaaggaatacacgaacatcttcctcaaatttggatctggctatgtaagtggctggggaagagtcttccacaaagggagatcagctttagttcttcagtaccttagagttccacttgttgaccgagccacatgtcttcgatctacaaagttcaccatctataacaacatgttctgtgctggcttccatgaaggaggtagagattcatgtcaaggagatagtgggggaccccatgttactgaagtggaagggaccagtttcttaactggaattattagctggggtgaagagtgtgcaatgaaaggcaaatatggaatatataccaaggtatcccggtatgtcaactggattaaggaaaaaacaaagctcacttaatgaaagatggatttccaaggttaattcattggaattgaaaattaacagggcctctcactaactaatcactttcccatcttttgttagatttgaatatatacattctatgatcattgctttttctctttacaggggagaatttcatattttacctgagcaaattgattagaaaatggaaccactagaggaatataatgtgttaggaaattacagtcatttctaagggcccagcccttgacaaaattgtgaagttaaattctccactctgtccatcagatactatggttctccactatggcaactaactcactcaattttccctccttagcagcattccatcttcccgatcttctttgcttctccaaccaaaacatcaatgtttattagttctgtatacagtacaggatctttggtctactctatcacaaggccagtaccacactcatgaagaaagaacacaggagtagctgagaggctaaaactcatcaaaaacactactccttttcctctaccctattcctcaatcttttaccttttccaaatcccaatccccaaatcagtttttctctttcttactccctctctcccttttaccctccatggtcgttaaaggagagatggggagcatcattctgttatacttctgtacacagttatacatgtctatcaaacccagacttgcttccatagtggggacttgcttttcagaacatagggatgaagtaaggtgcctgaaaagtttgggggaaaagtttctttcagagagttaagttattttatatatataatatatatataaaatatataatatacaatataaatatatagtgtgtgtgtgtatgcgtgtgtgtagacacacacgcatacacacatataatggaagcaataagccattctaagagcttgtatggttatggaggtctgactaggcatgatttgacgaaggcaagattggcatatcattgtaactaaaaaagctgacattgacccagacatattgtactctttctaaaaataataataataatgctaacagaaagaagagaaccgttcgtttgcaatctacagctagtagagactttgaggaagaattcaacagtgtgtcttcagcagtgttcagagccaagcaagaagttgaagttgcctagaccagaggacataagtatcatgtctcctttaactagcataccccgaagtggagaagggtgcagcaggctcaaaggcataagtcattccaatcagccaactaagttgtccttttctggtttcgtgttcaccatggaacattttgattatagttaatccttctatcttgaatcttctagagagttgctgaccaactgacgtatgtttccctttgtgaattaataaactggtgttctggttcataccttggctttttgtggattccattgatgtgaatcagtcaccctgtatttgatgatgcatgggactactgacaaaatcactctgactctgaccctgccaagctgctgccttctcctgccccaacctcacccccagccaggcctcactctttgctagttcctttagtcttttagtcaatatatttttgtcttcgcatataagtataaataaacatatttttaaatttctggctgggcccagtggctcacgcctataatc

SEQ ID NO: 6 - protein, 8 aa, Homo sapiens
  REGION 1..8: note = [CDS]:1129..1152 from SEQ ID NO 5
TEFWKQYV

SEQ ID NO: 7 - protein, 29 aa, Homo sapiens
  REGION 1..29: note = [CDS]:325..411 from SEQ ID NO 5
MQRVNMIMAESPGLITICLLGYLLSAECT

SEQ ID NO: 8 - protein, 38 aa, Homo sapiens
  REGION 1..38: note = [CDS]:1264..1377 from SEQ ID NO 5
DGDQCESNPCLNGGSCKDDINSYECWCPFGFEGKNCEL

SEQ ID NO: 9 - protein, 43 aa, Homo sapiens
  REGION 1..43: note = [CDS]:1582..1710 from SEQ ID NO 5
DVTCNIKNGRCEQFCKNSADNKVVCSCTEGYRLAENQKSCEPA

SEQ ID NO: 10 - protein, 55 aa, Homo sapiens
  REGION 1..55: note = [CDS]:776..940 from SEQ ID NO 5
VFLDHENANKILNRPKRYNSGKLEEFVQGNLERECMEEKCSFEEAREVFENTERT

SEQ ID NO: 11 - protein, 68 aa, Homo sapiens
  REGION 1..68: note = [CDS]:1881..2084 from SEQ ID NO 5
VPFPCGRVSVSQTSKLTRAEAVFPDVDYVNSTEAETILDNITQSTQSFNDFTRVVGGEDAKPGQFPWQ

SEQ ID NO: 12 - protein, 38 aa, Homo sapiens
  REGION 1..38: note = [CDS]:2303..2416 from SEQ ID NO 5
VVLNGKVDAFCGGSIVNEKWIVTAAHCVETGVKITVVA

SEQ ID NO: 13 - protein, 182 aa, Homo sapiens
  REGION 1..182: note = [CDS]:3085..3630 from SEQ ID NO 5
GEHNIEETEHTEQKRNVIRIIPHHNYNAAINKYNHDIALLELDEPLVLNSYVTPICIADKEYTNIFLKFGSGYVSGWGRVFHKGRSALVLQYLRVPLVDRATCLRSTKFTIYNNMFCAGFHEGGRDSCQGDSGGPHVTEVEGTSFLTGIISWGEECAMKGKYGIYTKVSRYVNWIKEKTKLT